European Patent Application EP 4 130 021 A1, published February 8, 2023. Title: Method of production of polymeric IgA-type antibody and multispecific polymeric IgA-type antibody. Applicant: TOKO YAKUHIN KOGYO CO., LTD. JAPAN as represented by DIRECTOR GENERAL of National Institute of Infectious Diseases. The sequence listing filed with the application follows.

SEQUENCE LISTING (16 sequences)

SEQ ID NO: 1 - protein, 353 aa, Homo sapiens
ASPTSPKVFPLSLCSTQPDGNVVIACLVQGFFPQEPLSVTWSESGQGVTARNFPPSQDASGDLYTTSSQLTLPATQCLAGKSVTCHVKHYTNPSQDVTVPCPVPSTPPTPSPSTPPTPSPSCCHPRLSLHRPALEDLLLGSEANLTCTLTGLRDASGVTFTWTPSSGKSAVQGPPERDLCGCYSVSSVLPGCAEPWNHGKTFTCTAAYPESKTPLTATLSKSGNTFRPEVHLLPPPSEELALNELVTLTCLARGFSPKDVLVRWLQGSQELPREKYLTWASRQEPSQGTTTFAVTSILRVAAEDWKKGDTFSCMVGHEALPLAFTQKTIDRLAGKPTHVNVSVVMAEVDGTCY

SEQ ID NO: 2 - protein, 340 aa, Homo sapiens
ASPTSPKVFPLSLDSTPQDGNVVVACLVQGFFPQEPLSVTWSESGQNVTARNFPPSQDASGDLYTTSSQLTLPATQCPDGKSVTCHVKHYTNSSQDVTVPCRVPPPPPCCHPRLSLHRPALEDLLLGSEANLTCTLTGLRDASGATFTWTPSSGKSAVQGPPERDLCGCYSVSSVLPGCAQPWNHGETFTCTAAHPELKTPLTANITKSGNTFRPEVHLLPPPSEELALNELVTLTCLARGFSPKDVLVRWLQGSQELPREKYLTWASRQEPSQGTTTYAVTSILRVAAEDWKKGETFSCMVGHEALPLAFTQKTIDRMAGKPTHINVSVVMAEADGTCY

SEQ ID NO: 3 - protein, 585 aa, Homo sapiens
KSPIFGPEEVNSVEGNSVSITCYYPPTSVNRHTRKYWCRQGARGGCITLISSEGYVSSKYAGRANLTNFPENGTFVVNIAQLSQDDSGRYKCGLGINSRGLSFDVSLEVSQGPGLLNDTKVYTVDLGRTVTINCPFKTENAQKRKSLYKQIGLYPVLVIDSSGYVNPNYTGRIRLDIQGTGQLLFSVVINQLRLSDAGQYLCQAGDDSNSNKKNADLQVLKPEPELVYEDLRGSVTFHCALGPEVANVAKFLCRQSSGENCDVVVNTLGKRAPAFEGRILLNPQDKDGSFSVVITGLRKEDAGRYLCGAHSDGQLQEGSPIQAWQLFVNEESTIPRSPTVVKGVAGGSVAVLCPYNRKESKSIKYWCLWEGAQNGRCPLLVDSEGWVKAQYEGRLSLLEEPGNGTFTVILNQLTSRDAGFYWCLTNGDTLWRTTVEIKIIEGEPNLKVPGNVTAVLGETLKVPCHFPCKFSSYEKYWCKWNNTGCQALPSQDEGPSKAFVNCDENSRLVSLTLNLVTRADEGWYWCGVKQGHFYGETAAVYVAVEERKAAGSRDVSLAKADAAPDEKVLDSGFREIENKAIQDPR

SEQ ID NO: 4 - protein, 224 aa, Artificial
  SC12
KSPIFGPEEVNSVEGNSVSITCYYPPTSVNRHTRKYWCRQGARGGCITLISSEGYVSSKYAGRANLTNFPENGTFVVNIAQLSQDDSGRYKCGLGINSRGLSFDVSLEVSQGPGLLNDTKVYTVDLGRTVTINCPFKTENAQKRKSLYKQIGLYPVLVIDSSGYVNPNYTGRIRLDIQGTGQLLFSVVINQLRLSDAGQYLCQAGDDSNSNKKNADLQVLKPEP

SEQ ID NO: 5 - protein, 618 aa, Artificial
  wild-type SC containing signal sequence, thrombin site, His tag
MLLFVLTCLLAVFPAISTKSPIFGPEEVNSVEGNSVSITCYYPPTSVNRHTRKYWCRQGARGGCITLISSEGYVSSKYAGRANLTNFPENGTFVVNIAQLSQDDSGRYKCGLGINSRGLSFDVSLEVSQGPGLLNDTKVYTVDLGRTVTINCPFKTENAQKRKSLYKQIGLYPVLVIDSSGYVNPNYTGRIRLDIQGTGQLLFSVVINQLRLSDAGQYLCQAGDDSNSNKKNADLQVLKPEPELVYEDLRGSVTFHCALGPEVANVAKFLCRQSSGENCDVVVNTLGKRAPAFEGRILLNPQDKDGSFSVVITGLRKEDAGRYLCGAHSDGQLQEGSPIQAWQLFVNEESTIPRSPTVVKGVAGGSVAVLCPYNRKESKSIKYWCLWEGAQNGRCPLLVDSEGWVKAQYEGRLSLLEEPGNGTFTVILNQLTSRDAGFYWCLTNGDTLWRTTVEIKIIEGEPNLKVPGNVTAVLGETLKVPCHFPCKFSSYEKYWCKWNNTGCQALPSQDEGPSKAFVNCDENSRLVSLTLNLVTRADEGWYWCGVKQGHFYGETAAVYVAVEERKAAGSRDVSLAKADAAPDEKVLDSGFREIENKAIQDPRKLLVPRGSPHHHHHH

SEQ ID NO: 6 - protein, 257 aa, Artificial
  SC12 containing signal sequence, thrombin site, His tag
MLLFVLTCLLAVFPAISTKSPIFGPEEVNSVEGNSVSITCYYPPTSVNRHTRKYWCRQGARGGCITLISSEGYVSSKYAGRANLTNFPENGTFVVNIAQLSQDDSGRYKCGLGINSRGLSFDVSLEVSQGPGLLNDTKVYTVDLGRTVTINCPFKTENAQKRKSLYKQIGLYPVLVIDSSGYVNPNYTGRIRLDIQGTGQLLFSVVINQLRLSDAGQYLCQAGDDSNSNKKNADLQVLKPEPKLLVPRGSPHHHHHH

SEQ ID NO: 7 - DNA, 1857 bp, Artificial
  wild-type SC containing signal sequence, thrombin site, His tag
atgctgctcttcgtgctcacctgcctgctggcggtcttcccagccatctccacgaagagtcccatatttggtcccgaggaggtgaatagtgtggaaggtaactcagtgtccatcacgtgctactacccacccacctctgtcaaccggcacacccggaagtactggtgccggcagggagctagaggtggctgcataaccctcatctcctcggagggctacgtctccagcaaatatgcaggcagggctaacctcaccaacttcccggagaacggcacatttgtggtgaacattgcccagctgagccaggatgactccgggcgctacaagtgtggcctgggcatcaatagccgaggcctgtcctttgatgtcagcctggaggtcagccagggtcctgggctcctaaatgacactaaagtctacacagtggacctgggcagaacggtgaccatcaactgccctttcaagactgagaatgctcaaaagaggaagtccttgtacaagcagataggcctgtaccctgtgctggtcatcgactccagtggttatgtaaatcccaactatacaggaagaatacgccttgatattcagggtactggccagttactgttcagcgttgtcatcaaccaactcaggctcagcgatgctgggcagtatctctgccaggctggggatgattccaatagtaataagaagaatgctgacctccaagtgctaaagcccgagcccgagctggtttatgaagacctgaggggctcagtgaccttccactgtgccctgggccctgaggtggcaaacgtggccaaatttctgtgccgacagagcagtggggaaaactgtgacgtggtcgtcaacaccctggggaagagggccccagcctttgagggcaggatcctgctcaacccccaggacaaggatggctcattcagtgtggtgatcacaggcctgaggaaggaggatgcagggcgctacctgtgtggagcccattcggatggtcagctgcaggaaggctcgcctatccaggcctggcaactcttcgtcaatgaggagtccacgattccccgcagccccactgtggtgaagggggtggcaggaggctctgtggccgtgctctgcccctacaaccgtaaggaaagcaaaagcatcaagtactggtgtctctgggaaggggcccagaatggccgctgccccctgctggtggacagcgaggggtgggttaaggcccagtacgagggccgcctctccctgctggaggagccaggcaacggcaccttcactgtcatcctcaaccagctcaccagccgggacgccggcttctactggtgtctgaccaacggcgatactctctggaggaccaccgtggagatcaagattatcgaaggagaaccaaacctcaaggtaccagggaatgtcacggctgtgctgggagagactctcaaggtcccctgtcactttccatgcaaattctcctcgtacgagaaatactggtgcaagtggaataacacgggctgccaggccctgcccagccaagacgaaggccccagcaaggccttcgtgaactgtgacgagaacagccggcttgtctccctgaccctgaacctggtgaccagggctgatgagggctggtactggtgtggagtgaagcagggccacttctatggagagactgcagccgtctatgtggcagttgaagagaggaaggcagcggggtcccgcgatgtcagcctagcgaaggcagacgctgctcctgatgagaaggtgctagactctggttttcgggagattgagaacaaagccattcaggatcccaggaagcttctggtgcctcgcggttcccctcaccaccaccaccaccactaa

SEQ ID NO: 8 - DNA, 774 bp, Artificial
  SC12 containing signal sequence, thrombin site, His tag
atgctgctcttcgtgctcacctgcctgctggcggtcttcccagccatctccacgaagagtcccatatttggtcccgaggaggtgaatagtgtggaaggtaactcagtgtccatcacgtgctactacccacccacctctgtcaaccggcacacccggaagtactggtgccggcagggagctagaggtggctgcataaccctcatctcctcggagggctacgtctccagcaaatatgcaggcagggctaacctcaccaacttcccggagaacggcacatttgtggtgaacattgcccagctgagccaggatgactccgggcgctacaagtgtggcctgggcatcaatagccgaggcctgtcctttgatgtcagcctggaggtcagccagggtcctgggctcctaaatgacactaaagtctacacagtggacctgggcagaacggtgaccatcaactgccctttcaagactgagaatgctcaaaagaggaagtccttgtacaagcagataggcctgtaccctgtgctggtcatcgactccagtggttatgtaaatcccaactatacaggaagaatacgccttgatattcagggtactggccagttactgttcagcgttgtcatcaaccaactcaggctcagcgatgctgggcagtatctctgccaggctggggatgattccaatagtaataagaagaatgctgacctccaagtgctaaagcccgagcccaagcttctggtgcctcgcggttcccctcaccaccaccaccaccactaa

SEQ ID NO: 9 - DNA, 390 bp, Homo sapiens
accggtgtacattcccaggtgcagctgcgggagtcgggcccaggactggtgaggccttcacagaccctgtccctcacctgcgttgtctctggtggctccatcaatcttggtaatgactactggaactggatccggcagcccgccgggaaggggctggagtgggttgggcgtatctattccagtgggagtgccaagtacaatccctccctcaagagtcgagtcaccatttcactagacacgtccaagaaccagttctccctggagctgacctccgtgaccgccgcagacacggccgtgtattactgtgcgagattttcggggagttaccaagatcatgatgcttttgatgtgtggggccaggggacaatggtcaccgtctcttcagctagc

SEQ ID NO: 10 - protein, 130 aa, Homo sapiens
TGVHSQVQLRESGPGLVRPSQTLSLTCVVSGGSINLGNDYWNWIRQPAGKGLEWVGRIYSSGSAKYNPSLKSRVTISLDTSKNQFSLELTSVTAADTAVYYCARFSGSYQDHDAFDVWGQGTMVTVSSAS

SEQ ID NO: 11 - DNA, 330 bp, Homo sapiens
accggtgtacattctgacatccagatgacccagtctccatcctccctgtctgcatctgtaggagacagagtcaccatcacttgccgggcgactcaggacattaacattggtttagcctggtatcagcaaaaaccagggaaagccccaaggctcctgctccattctgcgtccacattggagagtggggtcccatccaggttcagtggcagtggatctgggacggattacactctcaccatcagcagcctacagcctgaagattttgcaacttattactgtcaacaatatttcagttccccgtacacttttggccaggggaccaagctggag

SEQ ID NO: 12 - protein, 110 aa, Homo sapiens
TGVHSDIQMTQSPSSLSASVGDRVTITCRATQDINIGLAWYQQKPGKAPRLLLHSASTLESGVPSRFSGSGSGTDYTLTISSLQPEDFATYYCQQYFSSPYTFGQGTKLE

SEQ ID NO: 13 - DNA, 417 bp, Homo sapiens
accggtgtacattcccaggtgcagctgcaagagtcgggcccaggactggtgaagccttcggaaaccctgtccctcacctgcattgtctctgatgactccatcaggagttcctcctggagctgggtccggcagcccccagggaagggactggagtggattggaaatatctattacagtgggaccagcagcgacatcccctacagtgggagctccagttacaacccctccctcgagagtcgcgtcaccatgtcagtagacacgtccaagaaccagttctccctgacgctgagctctgtgaccgctgcggacacggccgtttattactgtgcgagacttactctgattcggggagttattcccccgtaccactttgactgctggggccagggaaccctggtcaccgtctcctcagctagc

SEQ ID NO: 14 - protein, 139 aa, Homo sapiens
TGVHSQVQLQESGPGLVKPSETLSLTCIVSDDSIRSSSWSWVRQPPGKGLEWIGNIYYSGTSSDIPYSGSSSYNPSLESRVTMSVDTSKNQFSLTLSSVTAADTAVYYCARLTLIRGVIPPYHFDCWGQGTLVTVSSAS

SEQ ID NO: 15 - DNA, 399 bp, Homo sapiens
accggttcctgggcccagtctgtgctgacgcagccgccctcagtgtctggggccccagggcagagggtcaccatctcctgcactgggagcagctccaacatcggggcagattatgatgtacattggtaccagcaatttccaggaacagcccccaaactcctcatctatggtaacaataatcggccctcaggggtccctgaccgattctctggctccaagtctggcacctcagcctccctggccatcactgggctccaggctgaggatgaggctgattattactgccagtcctatgacagcagcctgagtggtacctgggtgttcggcggagggaccaagctgaccgtcctaggtcagcccaaggctgccccctcggtcactctgttcccgccctcgagt

SEQ ID NO: 16 - protein, 133 aa, Homo sapiens
TGSWAQSVLTQPPSVSGAPGQRVTISCTGSSSNIGADYDVHWYQQFPGTAPKLLIYGNNNRPSGVPDRFSGSKSGTSASLAITGLQAEDEADYYCQSYDSSLSGTWVFGGGTKLTVLGQPKAAPSVTLFPPSS